European Patent Application EP 4 317 183 A1, published February 7, 2024. Title: KIT FOR DETECTING NEISSERIA GONORRHOEAE AND METHOD FOR DETECTING NEISSERIA GONORRHOEAE. Applicant: ASAHI KASEI KABUSHIKI KAISHA. The sequence listing filed with the application follows.

SEQUENCE LISTING (12 sequences)

SEQ ID NO: 1 - protein, 123 aa, Neisseria gonorrhoeae
MAITKEDILEAVGSLTVMELNDLVKAFEEKFGVSAAAVAVAGPAGAGAADAEEKTEFDVVLASAGDQKVGVIKVVRAITGLGLKEAKDIVDGAPKTIKEGVSKAEAEDIQKQLEAAGAKVEIK

SEQ ID NO: 2 - protein, 123 aa, Neisseria meningitidis
MAITKEDILEAVGSLTVMELNDLVKAFEEKFGVSAAAVAVAGPAGAGAADAEEKTEFDVVLASAGDQKVGVIKVVRAITGLGLKEAKDIVDGAPKTIKEGVSKAEAEDIQKQLEEAGAKVEIK

SEQ ID NO: 3 - protein, 121 aa, Escherichia coli
MSITKDQIIEAVAAMSVMDVVELISAMEEKFGVSAAAAVAVAAGPVEAAEEKTEFDVILKAAGANKVAVIKAVRGATGLGLKEAKDLVESAPAALKEGVSKDDAEALKKALEEAGAEVEVK

SEQ ID NO: 4 - protein, 110 aa, Artificial Sequence
  4
MLTVMELNDLVKAFEEKFGVSAAAVAVAGPAGAGAADAEEKTEFDVVLASAGDQKVGVIKVVRAITGLGLKEAKDIVDGAPKTIKEGVSKAEAEDIQKQLEAAGAKVEIK

SEQ ID NO: 5 - protein, 61 aa, Artificial Sequence
  5
MAGDQKVGVIKVVRAITGLGLKEAKDIVDGAPKTIKEGVSKAEAEDIQKQLEAAGAKVEIK

SEQ ID NO: 6 - protein, 101 aa, Artificial Sequence
  6
MAITKEDILEAVGSLTVMELNDLVKAFEEKFGVSAAAVAVAGPAGAGAADAEEKTEFDVVLASAGDQKVGVIKVVRAITGLGLKEAKDIVDGAPKTIKEGV

SEQ ID NO: 7 - protein, 114 aa, Artificial Sequence
  7
EVQLQQSGAELVKPGASVKLSCTASGFNIKDTYIYWVKQRPEQGLEWIGRIDPANGHTKCDPKFQGKATITSDTSSNTAYLQLNSLTSEDTAVYYCSKGYFHYWGQGTTLTVSS

SEQ ID NO: 8 - protein, 107 aa, Artificial Sequence
  8
DIQMTQSPSSLSASLGERVSLTCRASQEISGYLSWLQQKPDGTIKRLIYAASTLDSGVPKRFSGSRSGSDYSLTISSLESEDFADYYCQQYDSYPWTFGGGTKLEIK

SEQ ID NO: 9 - protein, 118 aa, Artificial Sequence
  9
EVQVQQSGPELVKPGASVKISCKASGYSFTDYYIHWVKQGHVKSLEWIGRIDPYNGASSYNQIFRDKASLTVDKSSSTAFMDLQSLTSDDSAVYYCARGHYGSGLAYWGQGTLVTVTA

SEQ ID NO: 10 - protein, 107 aa, Artificial Sequence
  10
DVQITQSPSYLAASPGETITINCKTNKSISKYLAWYQEKPGKTNKLLIYSGSTLQSGIPSRFSGSGSGTDFTLTISSLEPEDFAIYYCQQHNEFPLTFGAGTKLELK

SEQ ID NO: 11 - protein, 115 aa, Artificial Sequence
  11
DLVKPGASVKLSCKASGYTFTNYWINWIKQRPGQGLEWIGRIAPGSGSTYYNEMFKGKATLTVDTSSRTAYIQLSSLSSEDSAVYFCARFVTTVVAESYWYFDVWGAGTTVTVSS

SEQ ID NO: 12 - protein, 111 aa, Artificial Sequence
  12
DIVLTQSPASLSVSLGQRATISCRASESVEFFGTSLMQWYQQKPGQPPKLLISAASIVESGVPARFTGSGSGTDFSLNIHPVEEDDIAMYFCQQSRKVPWTFGGGTKLEIK